European Patent Application EP 4 123 027 A1, published January 25, 2023. Title: A method of mass production of target gene in plants. Applicant: POSTECH ACADEMY-INDUSTRY FOUNDATION. The sequence listing filed with the application follows.

SEQUENCE LISTING (10 sequences)

SEQ ID NO: 1 - DNA, 1220 bp, Artificial Sequence
  Mac promoter
agagatctcctttgccccagagatcacaatggacgacttcctctatctctacgatctagtcaggaagttcgacggagaaggtgacgataccatgttcaccactgataatgagaagattagccttttcaatttcagaaagaatgctaacccacagatggttagagaggcttacgcagcaggtctcatcaagacgatctacccgagcaataatctccaggagatcaaataccttcccaagaaggttaaagatgcagtcaaaagattcaggactaactgcatcaagaacacagagaaagatatatttctcaagatcagaagtactattccagtatggacgattcaaggcttgcttcacaaaccaaggcaagtaatagagattggagtctctaaaaaggtagttcccactgaatcaaaggccatggagtcaaagattcaaatagaggacctaacagaactcgccgtaaagactggcgaacagttcatacagagtctcttacgactcaatgacaagaagaaaatcttcgtcaacatggtggagcacgacacgcttgtctactccaaaaatatcaaagatacagtctcagaagaccaaagggcaattgagacttttcaacaaagggtaatatccggaaacctcctcggattccattgcccagctatctgtcactttattgtgaagatagtggaaaaggaaggtggctcctacaaatgccatcattgcgataaaggaaaggccatcgttgaagatgcctctgccgacagtggtcccaaagatggacccccacccacgaggagcatcgtggaaaaagaagacgttccaaccacgtcttcaaagcaagtggattgatgtgacgcaagacgtgacgtaagtatctgagctagtttttatttttctactaatttggtcgtttatttcggcgtgtaggacatggcaaccgggcctgaatttcgcgggtattctgtttctattccaactttttcttgatccgcagccattaacgacttttgaatagatacgctgacacgccaagcctcgctagtcaaaagtgtaccaaacaacgctttacagcaagaacggaatgcgcgtgacgctcgcggtgacgccatttcgccttttcagaaatggataaatagccttgcttcctattatatcttcccaaattaccaatacattacactagcatctgaatttcataaccaatctcgatacaccaaatcga

SEQ ID NO: 2 - DNA, 1220 bp, Artificial Sequence
  Mac T promoter
agagatctcctttgccccagagatcacaatggacgacttcctctatctctacgatctagtcaggaagttcgacggagaaggtgacgataccatgttcaccactgataatgagaagattagccttttcaatttcagaaagaatgctaacccacagatggttagagaggcttacgcagcaggtctcatcaagacgatctacccgagcaataatctccaggagatcaaataccttcccaagaaggttaaagatgcagtcaaaagattcaggactaactgcatcaagaacacagagaaagatatatttctcaagatcagaagtactattccagtatggacgattcaaggcttgcttcacaaaccaaggcaagtaatagagattggagtctctaaaaaggtagttcccactgaatcaaaggccatggagtcaaagattcaaatagaggacctaacagaactcgccgtaaagactggcgaacagttcatacagagtctcttacgactcaatgacaagaagaaaatcttcgtcaacatggtggagcacgacacgcttgtctactccaaaaatatcaaagatacagtctcagaagaccaaagggcaattgagacttttcaacaaagggtaatatccggaaacctcctcggattccattgcccagctatctgtcactttattgtgaagatagtggaaaaggaaggtggctcctacaaatgccatcattgcgataaaggaaaggccatcgttgaagatgcctctgccgacagtggtcccaaagatggacccccacccacgaggagcatcgtggaaaaagaagacgttccaaccacgtcttcaaagcaagtggattgatgtgacgcaagacgtgacgtaagtatctgagctagtttttatttttctactaatttggtcgtttatttcggcgtgtaggacatggcaaccgggcctgaatttcgcgggtattctgtttctattccaactttttcttgatccgcagccattaacgacttttgaatagatacgctgacacgccaagcctcgctagtcaaaagtgtaccaaacaacgctttacagcaagaacggaatgcgcgtgacgctcgcggtgacgccatttcgccttttcagaaatggataaatagccttgcttcctattatatcttcccaaattaccaatacattacactagcatctgaatttcataaccaatctcgatacaccaaatcgt

SEQ ID NO: 3 - DNA, 520 bp, Artificial Sequence
  RD29B terminator
aattttactcaaaatgttttggttgctatggtagggactatggggttttcggattccggtggaagtgagtggggaggcagtggcggaggtaagggagttcaagattctggaactgaagatttggggttttgcttttgaatgtttgcgtttttgtatgatgcctctgtttgtgaactttgatgtattttatctttgtgtgaaaaagagattgggttaataaaatatttgcttttttggataagaaactcttttagcggcccattaataaaggttacaaatgcaaaatcatgttagcgtcagatatttaattattcgaagatgattgtgatagatttaaaattatcctagtcaaaaagaaagagtaggttgagcagaaacagtgacatctgttgtttgtaccatacaaattagtttagattattggttaacatgttaaatggctatgcatgtgacatttagaccttatcggaattaatttgtagaattattaattaagatgttgattagttcaaacaaaaat

SEQ ID NO: 4 - DNA, 1025 bp, Artificial Sequence
  BiP-sGFP-HDEL
atggctcgctcgtttggagctaacagtaccgttgtgttggcgatcatcttcttcggtgagtgattttccgatcttcttctccgatttagatctcctctacattgttgcttaatctcagaaccttttttcgttgttcctggatctgaatgtgtttgtttgcaatttcacgatcttaaaaggttagatctcgattggtattgacgattggaatctttacgatttcaggatgtttatttgcgttgtcctctgcaatagaagaggctacgaagttaaggatccaagatgatgatgataaggtgagcaagggcgaggagctgttcaccggggtggtgcccatcctggtcgagctggacggcgacgtaaacggccacaagttcagcgtgtccggcgagggcgagggcgatgccacctacggcaagctgaccctgaagttcatctgcaccaccggcaagctgcccgtgccctggcccaccctcgtgaccaccttcacctacggcgtgcagtgcttcagccgctaccccgaccacatgaagcagcacgacttcttcaagtccgccatgcccgaaggctacgtccaggagcgcaccatcttcttcaaggacgacggcaactacaagacccgcgccgaggtgaagttcgagggcgacaccctggtgaaccgcatcgagctgaagggcatcgacttcaaggaggacggcaacatcctggggcacaagctggagtacaactacaacagccacaacgtctatatcatggccgacaagcagaagaacggcatcaaggtgaacttcaagatccgccacaacatcgaggacggcagcgtgcagctcgccgaccactaccagcagaacacccccatcggcgacggccccgtgctgctgcccgacaaccactacctgagcacccagtccgccctgagcaaagaccccaacgagaagcgcgatcacatggtcctgctggagttcgtgaccgccgccgggatcactctcggcatggacgagctgtacaagcacgatgagctctag

SEQ ID NO: 5 - DNA, 272 bp, Artificial Sequence
  BiP
atggctcgctcgtttggagctaacagtaccgttgtgttggcgatcatcttcttcggtgagtgattttccgatcttcttctccgatttagatctcctctacattgttgcttaatctcagaaccttttttcgttgttcctggatctgaatgtgtttgtttgcaatttcacgatcttaaaaggttagatctcgattggtattgacgattggaatctttacgatttcaggatgtttatttgcgttgtcctctgcaatagaagaggctacgaagtta

SEQ ID NO: 6 - DNA, 21 bp, Artificial Sequence
  5' UTR, M
ggcgtgtgtgtgtgttaaaga

SEQ ID NO: 7 - DNA, 714 bp, Artificial Sequence
  sGFP
gtgagcaagggcgaggagctgttcaccggggtggtgcccatcctggtcgagctggacggcgacgtaaacggccacaagttcagcgtgtccggcgagggcgagggcgatgccacctacggcaagctgaccctgaagttcatctgcaccaccggcaagctgcccgtgccctggcccaccctcgtgaccaccttcacctacggcgtgcagtgcttcagccgctaccccgaccacatgaagcagcacgacttcttcaagtccgccatgcccgaaggctacgtccaggagcgcaccatcttcttcaaggacgacggcaactacaagacccgcgccgaggtgaagttcgagggcgacaccctggtgaaccgcatcgagctgaagggcatcgacttcaaggaggacggcaacatcctggggcacaagctggagtacaactacaacagccacaacgtctatatcatggccgacaagcagaagaacggcatcaaggtgaacttcaagatccgccacaacatcgaggacggcagcgtgcagctcgccgaccactaccagcagaacacccccatcggcgacggccccgtgctgctgcccgacaaccactacctgagcacccagtccgccctgagcaaagaccccaacgagaagcgcgatcacatggtcctgctggagttcgtgaccgccgccgggatcactctcggcatggacgagctgtacaag

SEQ ID NO: 8 - DNA, 12 bp, Artificial Sequence
  HDEL
cacgatgagctc

SEQ ID NO: 9 - DNA, 1056 bp, Artificial Sequence
  P38
atggaaaatgatcctagagtccggaagttcgcatctgatggcgcccaatgggcgataaagtggcagaagaagggctggtcaaccctaaccagcagacagaaacagaccgcccgcgcagcgatggggatcaagctctctcctgtggcgcaacctgtgcagaaagtgactcgactgagtgctccggtggcccttgcctaccgcgaggttaccacccagcctcgggtctctactgccagggacggcataaccagaagcggttctgaactgatcacaaccttgaagaagaacactgacactgaacctaagtacaccacagctgtgcttaacccaagcgaacccggaacattcaaccagctcattaaggaggcggcccagtatgaaaaataccgattcacgtcactcagatttaggtactcccccatgagcccttcaaccaccggaggcaaggtggctctggcattcgatcgagatgccgccaaacctccgcccaacgacctcgcttccctctacaacatagagggttgtgtatctagcgtgccctggacagggtttattttgaccgtcccaacagattctactgaccgctttgtggcggatggtatcagcgatccaaagcttgtcgatttcggcaagcttatcatggccacctacggccaaggagccaatgatgccgcccaactcggtgaagtgcgagtcgagtacaccgtgcagctcaagaacagaactggctcaaccagcgacgcccagattggggacttcgcaggtgttaaggacggacccaggctggtttcatggtccaagaccaaggggacagctgggtgggagcacgattgtcattttctcggaaccggaaacttctcgttgacattgttctacgagaaggcgccggtctcggggctagaaaacgcagacgcctctgacttctcggtcctgggagaagccgcagcaggtagtgtccaatgggcaggagtgaaggtagcagaaaggggacaaggcgtgaaaatggtcacaactgaggagcagccaaagggtaaatggcaagcactcagaatttag

SEQ ID NO: 10 - DNA, 21 bp, Artificial Sequence
  L 5'-UTR
attattacatcaaaacaaaaa